European Patent Application EP 4 467 139 A1, published November 27, 2024. Title: ZAK ALPHA KINASE (MAP3K20) INHIBITORS FOR USE IN THE TREATMENT OF ANEMIA. Applicant: Universidad de Murcia. The sequence listing filed with the application follows.

SEQUENCE LISTING (9 sequences)

SEQ ID NO: 1 - DNA, 21 bp, synthetic construct
  source 1..21: mol_type = other DNA
tgagcctgactgagctcttga

SEQ ID NO: 2 - DNA, 21 bp, synthetic construct
  source 1..21: mol_type = other DNA
agccagtcctggttacactct

SEQ ID NO: 3 - DNA, 24 bp, synthetic construct
  source 1..24: mol_type = other DNA
ttggccatcatttaatggacccgt

SEQ ID NO: 4 - DNA, 21 bp, synthetic construct
  source 1..21: mol_type = other DNA
ttttggttcagtcgcccagca

SEQ ID NO: 5 - DNA, 23 bp, synthetic construct
  source 1..23: mol_type = other DNA
gtgtgggattcctctgcatctta

SEQ ID NO: 6 - DNA, 21 bp, synthetic construct
  source 1..21: mol_type = other DNA
atgcagcttttgggtgacgta

SEQ ID NO: 7 - DNA, 20 bp, synthetic construct
  source 1..20: mol_type = other DNA
tcacagaagactcaactagc

SEQ ID NO: 8 - DNA, 20 bp, synthetic construct
  source 1..20: mol_type = other DNA
aagcccctccagacctttga

SEQ ID NO: 9 - DNA, 20 bp, synthetic construct
  source 1..20: mol_type = other DNA
ggtcccacaggataaagaag